European Patent Application EP 4 524 239 A1, published March 19, 2025. Title: 生理活性物質を含有する細胞外小胞を生産する方法. Applicant: 国立大学法人　東京大学. Application JP. The sequence listing filed with the application follows.

SEQUENCE LISTING (6 sequences)

SEQ ID NO: 1 - DNA, 33 bp, synthetic construct
  misc_feature 1..33: note = Synthetic primer
  source 1..33: mol_type = other DNA
accgtcgaccatggtgctgctgctggccagatg

SEQ ID NO: 2 - DNA, 33 bp, synthetic construct
  misc_feature 1..33: note = Synthetic primer
  source 1..33: mol_type = other DNA
caaggatcccggccgccggatttggccgccacg

SEQ ID NO: 3 - DNA, 36 bp, synthetic construct
  misc_feature 1..36: note = Synthetic primer
  source 1..36: mol_type = other DNA
accctcgagctatgcctgaggaaacccagacccaag

SEQ ID NO: 4 - DNA, 39 bp, synthetic construct
  misc_feature 1..39: note = Synthetic primer
  source 1..39: mol_type = other DNA
accggtaccttagtctacttcttccatgcgtgatgtgtc

SEQ ID NO: 5 - DNA, 37 bp, synthetic construct
  misc_feature 1..37: note = Synthetic primer
  source 1..37: mol_type = other DNA
tccgaattccatggacgaggacgtgctgaccactctg

SEQ ID NO: 6 - DNA, 42 bp, synthetic construct
  misc_feature 1..42: note = Synthetic primer
  source 1..42: mol_type = other DNA
aatgcggccgcctatagcacagagcagtaaccgccgcaggcg